European Patent Application EP 4 790 067 A1, published August 12, 2026. Title: O6-벤질구아닌 결합 단백질을 포함하는 키메라 어댑터 단백질 및 이를 포함하는 세포외 소포체. Applicant: 재단법인 대구경북과학기술원. The sequence listing filed with the application follows.

SEQUENCE LISTING (12 sequences)

SEQ ID NO: 1 - protein, 605 aa, synthetic construct
MDKDCEMKRTTLDSPLGKLELSGCEQGLHRIIFLGKGTSAADAVEVPAPAAVLGGPEPLMQATAWLNAYFHQPEAIEEFPVPALHHPVFQQESFTRQVLWKLLKVVKFGEVISYSHLAALAGNPAATAAVKTALSGNPVPILIPCHRVVQGDLDVGGYEGGLAVKEWLLAHEGHRLGKPGLGGSEAAAKEAAAKEAAAKEAAAKEAAAKEAAAKEAAAKEAAAKGSTSGSGKPGSGEGSTKGGSAVGQDTQEVIVVPHSLPFKVVVISAILALVVLTIISLIILIMLWQKKPRGGGGSMVSKGEELFTGVVPILVELDGDVNGHKFSVSGEGEGDATYGKLTLKFICTTGKLPVPWPTLVTTLTYGVQCFSRYPDHMKQHDFFKSAMPEGYVQERTIFFKDDGNYKTRAEVKFEGDTLVNRIELKGIDFKEDGNILGHKLEYNYNSHNVYIMADKQKNGIKVNFKIRHNIEDGSVQLADHYQQNTPIGDGPVLLPDNHYLSTQSALSKDPNEKRDHMVLLEFVTAAGITLGMDELYKGGGGSSLYPSLEDLKVDKVIQAQTAFSANPANPAILSEASAPIPHDGNLYPRLYPELSQYMGLSLEGG

SEQ ID NO: 2 - protein, 182 aa, synthetic construct
MDKDCEMKRTTLDSPLGKLELSGCEQGLHRIIFLGKGTSAADAVEVPAPAAVLGGPEPLMQATAWLNAYFHQPEAIEEFPVPALHHPVFQQESFTRQVLWKLLKVVKFGEVISYSHLAALAGNPAATAAVKTALSGNPVPILIPCHRVVQGDLDVGGYEGGLAVKEWLLAHEGHRLGKPGLG

SEQ ID NO: 3 - protein, 40 aa, synthetic construct
EAAAKEAAAKEAAAKEAAAKEAAAKEAAAKEAAAKEAAAK

SEQ ID NO: 4 - protein, 49 aa, synthetic construct
AVGQDTQEVIVVPHSLPFKVVVISAILALVVLTIISLIILIMLWQKKPR

SEQ ID NO: 5 - protein, 239 aa, synthetic construct
MVSKGEELFTGVVPILVELDGDVNGHKFSVSGEGEGDATYGKLTLKFICTTGKLPVPWPTLVTTLTYGVQCFSRYPDHMKQHDFFKSAMPEGYVQERTIFFKDDGNYKTRAEVKFEGDTLVNRIELKGIDFKEDGNILGHKLEYNYNSHNVYIMADKQKNGIKVNFKIRHNIEDGSVQLADHYQQNTPIGDGPVLLPDNHYLSTQSALSKDPNEKRDHMVLLEFVTAAGITLGMDELYK

SEQ ID NO: 6 - protein, 63 aa, synthetic construct
SLYPSLEDLKVDKVIQAQTAFSANPANPAILSEASAPIPHDGNLYPRLYPELSQYMGLSLEGG

SEQ ID NO: 7 - DNA, 1815 bp, synthetic construct
  source 1..1815: mol_type = other DNA
atggacaaagactgcgaaatgaagcgcaccaccctggatagccctctgggcaagctggaactgtctgggtgcgaacagggcctgcaccgtatcatcttcctgggcaaaggaacatctgccgccgacgccgtggaagtgcctgccccagccgccgtgctgggcggaccagagccactgatgcaggccaccgcctggctcaacgcctactttcaccagcctgaggccatcgaggagttccctgtgccagccctgcaccacccagtgttccagcaggagagctttacccgccaggtgctgtggaaactgctgaaagtggtgaagttcggagaggtcatcagctacagccacctggccgccctggccggcaatcccgccgccaccgccgccgtgaaaaccgccctgagcggaaatcccgtgcccattctgatcccctgccaccgggtggtgcagggcgacctggacgtggggggctacgagggcgggctcgccgtgaaagagtggctgctggcccacgagggccacagactgggcaagcctgggctgggtggctccgaagccgctgctaaggaagccgctgctaaggaagccgctgctaaggaagccgctgctaaggaagccgctgctaaggaagccgctgctaaggaagccgctgctaaggaagccgctgctaagggctccaccagcggcagcggcaagccaggctccggcgaaggcagcaccaaaggcggatccgctgtgggccaggacacgcaggaggtcatcgtggtgccacactccttgccctttaaggtggtggtgatctcagccatcctggccctggtggtgctcaccatcatctcccttatcatcctcatcatgctttggcagaagaagccacgtggcggtggcggttccatggtgagcaagggcgaggagctgttcaccggggtggtgcccatcctggtcgagctggacggcgacgtaaacggccacaagttcagcgtgtccggcgagggcgagggcgatgccacctacggcaagctgaccctgaagttcatctgcaccaccggcaagctgcccgtgccctggcccaccctcgtgaccaccctgacctacggcgtgcagtgcttcagccgctaccccgaccacatgaagcagcacgacttcttcaagtccgccatgcccgaaggctacgtccaggagcgcaccatcttcttcaaggacgacggcaactacaagacccgcgccgaggtgaagttcgagggcgacaccctggtgaaccgcatcgagctgaagggcatcgacttcaaggaggacggcaacatcctggggcacaagctggagtacaactacaacagccacaacgtctatatcatggccgacaagcagaagaacggcatcaaggtgaacttcaagatccgccacaacatcgaggacggcagcgtgcagctcgccgaccactaccagcagaacacccccatcggcgacggccccgtgctgctgcccgacaaccactacctgagcacccagtccgccctgagcaaagaccccaacgagaagcgcgatcacatggtcctgctggagttcgtgaccgccgccgggatcactctcggcatggacgagctgtacaagggcggtggcggttcctctctctatccatctctcgaagacttgaaggtagacaaagtaattcaggctcaaactgctttttctgcaaaccctgccaatccagcaattttgtcagaagcttctgctcctatccctcacgatggaaatctctatcccagactgtatccagagctctctcaatacatggggctgagtttagaaggcggt

SEQ ID NO: 8 - DNA, 546 bp, synthetic construct
  source 1..546: mol_type = other DNA
atggacaaagactgcgaaatgaagcgcaccaccctggatagccctctgggcaagctggaactgtctgggtgcgaacagggcctgcaccgtatcatcttcctgggcaaaggaacatctgccgccgacgccgtggaagtgcctgccccagccgccgtgctgggcggaccagagccactgatgcaggccaccgcctggctcaacgcctactttcaccagcctgaggccatcgaggagttccctgtgccagccctgcaccacccagtgttccagcaggagagctttacccgccaggtgctgtggaaactgctgaaagtggtgaagttcggagaggtcatcagctacagccacctggccgccctggccggcaatcccgccgccaccgccgccgtgaaaaccgccctgagcggaaatcccgtgcccattctgatcccctgccaccgggtggtgcagggcgacctggacgtggggggctacgagggcgggctcgccgtgaaagagtggctgctggcccacgagggccacagactgggcaagcctgggctgggt

SEQ ID NO: 9 - DNA, 120 bp, synthetic construct
  source 1..120: mol_type = other DNA
gaagccgctgctaaggaagccgctgctaaggaagccgctgctaaggaagccgctgctaaggaagccgctgctaaggaagccgctgctaaggaagccgctgctaaggaagccgctgctaag

SEQ ID NO: 10 - DNA, 147 bp, synthetic construct
  source 1..147: mol_type = other DNA
gctgtgggccaggacacgcaggaggtcatcgtggtgccacactccttgccctttaaggtggtggtgatctcagccatcctggccctggtggtgctcaccatcatctcccttatcatcctcatcatgctttggcagaagaagccacgt

SEQ ID NO: 11 - DNA, 717 bp, synthetic construct
  source 1..717: mol_type = other DNA
atggtgagcaagggcgaggagctgttcaccggggtggtgcccatcctggtcgagctggacggcgacgtaaacggccacaagttcagcgtgtccggcgagggcgagggcgatgccacctacggcaagctgaccctgaagttcatctgcaccaccggcaagctgcccgtgccctggcccaccctcgtgaccaccctgacctacggcgtgcagtgcttcagccgctaccccgaccacatgaagcagcacgacttcttcaagtccgccatgcccgaaggctacgtccaggagcgcaccatcttcttcaaggacgacggcaactacaagacccgcgccgaggtgaagttcgagggcgacaccctggtgaaccgcatcgagctgaagggcatcgacttcaaggaggacggcaacatcctggggcacaagctggagtacaactacaacagccacaacgtctatatcatggccgacaagcagaagaacggcatcaaggtgaacttcaagatccgccacaacatcgaggacggcagcgtgcagctcgccgaccactaccagcagaacacccccatcggcgacggccccgtgctgctgcccgacaaccactacctgagcacccagtccgccctgagcaaagaccccaacgagaagcgcgatcacatggtcctgctggagttcgtgaccgccgccgggatcactctcggcatggacgagctgtacaag

SEQ ID NO: 12 - DNA, 189 bp, synthetic construct
  source 1..189: mol_type = other DNA
tctctctatccatctctcgaagacttgaaggtagacaaagtaattcaggctcaaactgctttttctgcaaaccctgccaatccagcaattttgtcagaagcttctgctcctatccctcacgatggaaatctctatcccagactgtatccagagctctctcaatacatggggctgagtttagaaggcggt